European Patent Application EP 4 223 878 A1, published August 9, 2023. Title: SARS-CoV-2 binding peptide. Applicant: EPSILON MOLECULAR ENGINEERING, INC. THE KITASATO INSTITUTE KAO CORPORATION. The sequence listing filed with the application follows.

SEQUENCE LISTING (111 sequences)

SEQ ID NO: 1 - protein, 14 aa, Artificial Sequence
  Designed peptide
LLRRYNYGFTFDNY

SEQ ID NO: 2 - protein, 10 aa, Artificial Sequence
  Designed peptide
FGGSDFLMDY

SEQ ID NO: 3 - protein, 10 aa, Artificial Sequence
  Designed peptide
AWSDYEYLEV

SEQ ID NO: 4 - protein, 10 aa, Artificial Sequence
  Designed peptide
TPWYSASHTY

SEQ ID NO: 5 - protein, 8 aa, Artificial Sequence
  Designed peptide
VTWLRGDY

SEQ ID NO: 6 - protein, 14 aa, Artificial Sequence
  Designed peptide
ITTGSPLLGGGMDF

SEQ ID NO: 7 - protein, 8 aa, Artificial Sequence
  Designed peptide
VFPSGGDY

SEQ ID NO: 8 - protein, 11 aa, Artificial Sequence
  Designed peptide
VGLFGIQASDY

SEQ ID NO: 9 - protein, 13 aa, Artificial Sequence
  Designed peptide
PGVVTGSYDVRNY

SEQ ID NO: 10 - protein, 10 aa, Artificial Sequence
  Designed peptide
GFAFSSYPMY

SEQ ID NO: 11 - protein, 10 aa, Artificial Sequence
  Designed peptide
RRTSSTYAMG

SEQ ID NO: 12 - protein, 10 aa, Artificial Sequence
  Designed peptide
APTFMTYTMA

SEQ ID NO: 13 - protein, 10 aa, Artificial Sequence
  Designed peptide
GFTFTTYAMT

SEQ ID NO: 14 - protein, 10 aa, Artificial Sequence
  Designed peptide
DQIFDNYNMA

SEQ ID NO: 15 - protein, 10 aa, Artificial Sequence
  Designed peptide
GRTWNIASMT

SEQ ID NO: 16 - protein, 10 aa, Artificial Sequence
  Designed peptide
GRTFSSCAMG

SEQ ID NO: 17 - protein, 10 aa, Artificial Sequence
  Designed peptide
GQTFSSYNMA

SEQ ID NO: 18 - protein, 10 aa, Artificial Sequence
  Designed peptide
GTIFSTNAMS

SEQ ID NO: 19 - protein, 10 aa, Artificial Sequence
  Designed peptide
FIDGEGTSTS

SEQ ID NO: 20 - protein, 10 aa, Artificial Sequence
  Designed peptide
AISWDGGRTY

SEQ ID NO: 21 - protein, 10 aa, Artificial Sequence
  Designed peptide
ALSKNFVTTS

SEQ ID NO: 22 - protein, 10 aa, Artificial Sequence
  Designed peptide
TISGADGSTY

SEQ ID NO: 23 - protein, 10 aa, Artificial Sequence
  Designed peptide
ALSWGDSNTG

SEQ ID NO: 24 - protein, 11 aa, Artificial Sequence
  Designed peptide
TIKWSDLATYY

SEQ ID NO: 25 - protein, 10 aa, Artificial Sequence
  Designed peptide
AISRGGGSTS

SEQ ID NO: 26 - protein, 10 aa, Artificial Sequence
  Designed peptide
TISWGGGSTG

SEQ ID NO: 27 - protein, 9 aa, Artificial Sequence
  Designed peptide
AITSGGNTN

SEQ ID NO: 28 - protein, 25 aa, Artificial Sequence [sequence omitted]

SEQ ID NO: 29 - protein, 25 aa, Artificial Sequence
  Designed peptide
EVQLVESGGGLVQAGDSLRLSCAAT

SEQ ID NO: 30 - protein, 25 aa, Artificial Sequence
  Designed peptide
EVQLVESGGGFVQAGGSLRLSCRVS

SEQ ID NO: 31 - protein, 25 aa, Artificial Sequence
  Designed peptide
EVQLVESGGDVVQPGGSLRLSCAAS

SEQ ID NO: 32 - protein, 25 aa, Artificial Sequence
  Designed peptide
EVQLVESGGGLVQAGGSLRLSCTAS

SEQ ID NO: 33 - protein, 25 aa, Artificial Sequence
  Designed peptide
EVQLVESGGGLVQAGDSLRLSCTAS

SEQ ID NO: 34 - protein, 25 aa, Artificial Sequence
  Designed peptide
EVQLVESGGGLVQPGGSLTLSCAAS

SEQ ID NO: 35 - protein, 14 aa, Artificial Sequence
  Designed peptide
WVRQAPGKGLEWIS

SEQ ID NO: 36 - protein, 14 aa, Artificial Sequence
  Designed peptide
WFRQAPGKGLEWVA

SEQ ID NO: 37 - protein, 14 aa, Artificial Sequence
  Designed peptide
WFRQAPGNEREFVA

SEQ ID NO: 38 - protein, 14 aa, Artificial Sequence
  Designed peptide
WVRQAPGEGLEAVS

SEQ ID NO: 39 - protein, 14 aa, Artificial Sequence
  Designed peptide
WFRQSPGKEREFVA

SEQ ID NO: 40 - protein, 15 aa, Artificial Sequence
  Designed peptide
WFRQAPGGKERTFVA

SEQ ID NO: 41 - protein, 14 aa, Artificial Sequence
  Designed peptide
WFRQAPGKEREFVA

SEQ ID NO: 42 - protein, 14 aa, Artificial Sequence
  Designed peptide
WYRQAPGKQRELVA

SEQ ID NO: 43 - protein, 39 aa, Artificial Sequence
  Designed peptide
YADSVKGRFTISRDNAKNTVYLQMNSLKPEDTAVYYCNA

SEQ ID NO: 44 - protein, 39 aa, Artificial Sequence
  Designed peptide
YAESVKGRFTISRDNAKNTVYLQMNSLKPEDTAVYYCYS

SEQ ID NO: 45 - protein, 39 aa, Artificial Sequence
  Designed peptide
YADSVKGRFTISRDNAKNTVYLQMNSLKPEDTAVYYCNV

SEQ ID NO: 46 - protein, 39 aa, Artificial Sequence
  Designed peptide
YADSVKGRFTISRDNANNTVYLQMNSLKPEDTAVYYCAA

SEQ ID NO: 47 - protein, 39 aa, Artificial Sequence
  Designed peptide
YADSVKGRFTISRDNAKNTVYLQMNSLKPEDTAVYYCYA

SEQ ID NO: 48 - protein, 38 aa, Artificial Sequence
  Designed peptide
TDSVKGRFTISRGNSKNTVYLQMNSLKPEDTGVYFCYA

SEQ ID NO: 49 - protein, 39 aa, Artificial Sequence
  Designed peptide
YADSVKGRFTISKDRARNTAYLEMNSLKPEDTAIYYCYA

SEQ ID NO: 50 - protein, 39 aa, Artificial Sequence
  Designed peptide
YADSVKGRFTISRDHAKNTVYLQMKDLKPEDTGAYYCYL

SEQ ID NO: 51 - protein, 11 aa, Artificial Sequence
  Designed peptide
WGQGTQVTVSS

SEQ ID NO: 52 - protein, 11 aa, Artificial Sequence
  Designed peptide
WGQGTLVTVSS

SEQ ID NO: 53 - protein, 11 aa, Artificial Sequence
  Designed peptide
WGKGTLVTVSS

SEQ ID NO: 54 - DNA, 117 bp, Artificial Sequence
  Synthetic oligonucleotide
gatcccgcgaaattaatacgactcactataggggaagtatttttacaacaattaccaacaacaacaacaaacaacaacaacattacattttacattctacaactacaagccaccatg

SEQ ID NO: 55 - DNA, 61 bp, Artificial Sequence
  Synthetic oligonucleotide
tttccacgccgccccccgtcctgcttccgccgtgatgatgatgatgatggctgcctccccc

SEQ ID NO: 56 - DNA, 117 bp, Artificial Sequence; identical to SEQ ID NO: 54
  Synthetic oligonucleotide

SEQ ID NO: 57 - DNA, 61 bp, Artificial Sequence; identical to SEQ ID NO: 55
  Synthetic oligonucleotide

SEQ ID NO: 58 - DNA, 60 bp, Artificial Sequence
  Synthetic oligonucleotide
gatcccgcgaaattaatacgactcactataggggaagtatttttacaacaattaccaaca

SEQ ID NO: 59 - DNA, 22 bp, Artificial Sequence
  Synthetic oligonucleotide
tttccacgccgccccccgtcct

SEQ ID NO: 60 - DNA, 58 bp, Artificial Sequence
  Synthetic oligonucleotide
  misc_feature (34)..(37): n is a, c, g, or t
tcgtcggcagcgtcagatgtgtataagagacagnnnnatggctgaggtgcagctcgtg

SEQ ID NO: 61 - DNA, 63 bp, Artificial Sequence
  Synthetic oligonucleotide
  misc_feature (35)..(38): n is a, c, g, or t
gtctcgtgggctcggagatgtgtataagagacagnnnntgatgatgatggctaccacctcccg

SEQ ID NO: 62 - DNA, 33 bp, Artificial Sequence
  Synthetic oligonucleotide
gatcccgcgaaattaatacgactcactataggg

SEQ ID NO: 63 - DNA, 106 bp, Artificial Sequence
  Synthetic oligonucleotide
gaaattaatacgactcactatagggagaccacaacggtttccctctagaaataattttgtttaactttaagaaggagatataccaatggctgaggtgcagctcgtg

SEQ ID NO: 64 - DNA, 72 bp, Artificial Sequence
  Synthetic oligonucleotide
ccgccgtgatgatgttacttacttacttgtcgtcatcgtctttgtagtcgtgatgatgatgatgatggctgc

SEQ ID NO: 65 - protein, 123 aa, Artificial Sequence
  Designed peptide
EVQLVESGGGLVQPGGSLRLSCAASGFAFSSYPMYWVRQAPGKGLEWISFIDGEGTSTSYADSVKGRFTISRDNAKNTVYLQMNSLKPEDTAVYYCNALLRRYNYGFTFDNYWGQGTQVTVSS

SEQ ID NO: 66 - protein, 119 aa, Artificial Sequence
  Designed peptide
EVQLVESGGGLVQAGDSLRLSCAATRRTSSTYAMGWFRQAPGKGLEWVAAISWDGGRTYYAESVKGRFTISRDNAKNTVYLQMNSLKPEDTAVYYCYSFGGSDFLMDYWGQGTQVTVSS

SEQ ID NO: 67 - protein, 119 aa, Artificial Sequence
  Designed peptide
EVQLVESGGGFVQAGGSLRLSCRVSAPTFMTYTMAWFRQAPGNEREFVAALSKNFVTTSYADSVKGRFTISRDNAKNTVYLQMNSLKPEDTAVYYCNVAWSDYEYLEVWGQGTLVTVSS

SEQ ID NO: 68 - protein, 119 aa, Artificial Sequence
  Designed peptide
EVQLVESGGDVVQPGGSLRLSCAASGFTFTTYAMTWVRQAPGEGLEAVSTISGADGSTYYADSVKGRFTISRDNANNTVYLQMNSLKPEDTAVYYCAATPWYSASHTYWGQGTQVTVSS

SEQ ID NO: 69 - protein, 117 aa, Artificial Sequence
  Designed peptide
EVQLVESGGGLVQAGGSLRLSCTASDQIFDNYNMAWFRQSPGKEREFVAALSWGDSNTGYADSVKGRFTISRDNAKNTVYLQMNSLKPEDTAVYYCYAVTWLRGDYWGQGTQVTVSS

SEQ ID NO: 70 - protein, 124 aa, Artificial Sequence
  Designed peptide
EVQLVESGGGLVQAGGSLRLSCTASGRTWNIASMTWFRQAPGGKERTFVATIKWSDLATYYTDSVKGRFTISRGNSKNTVYLQMNSLKPEDTGVYFCYAITTGSPLLGGGMDFWGKGTLVTVSS

SEQ ID NO: 71 - protein, 117 aa, Artificial Sequence
  Designed peptide
EVQLVESGGGLVQAGDSLRLSCTASGRTFSSCAMGWFRQAPGKEREFVAAISRGGGSTSYADSVKGRFTISKDRARNTAYLEMNSLKPEDTAIYYCYAVFPSGGDYWGQGTQVTVSS

SEQ ID NO: 72 - protein, 120 aa, Artificial Sequence
  Designed peptide
EVQLVESGGGLVQPGGSLTLSCAASGQTFSSYNMAWFRQSPGKEREFVATISWGGGSTGYADSVKGRFTISRDHAKNTVYLQMKDLKPEDTGAYYCYLVGLFGIQASDYWGQGTQVTVSS

SEQ ID NO: 73 - protein, 121 aa, Artificial Sequence
  Designed peptide
EVQLVESGGGLVQPGGSLRLSCAASGTIFSTNAMSWYRQAPGKQRELVAAITSGGNTNYADSVKGRFTISRDNAKNTVYLQMNSLKPEDTAVYYCNAPGVVTGSYDVRNYWGQGTQVTVSS

SEQ ID NO: 74 - protein, 10 aa, Artificial Sequence
  Designed peptide
GGGSHHHHHH

SEQ ID NO: 75 - DNA, 15 bp, Artificial Sequence
  Synthetic oligonucleotide
gcagctcttgcagca

SEQ ID NO: 76 - DNA, 15 bp, Artificial Sequence
  Synthetic oligonucleotide
tctattaaactagtt

SEQ ID NO: 77 - DNA, 426 bp, Artificial Sequence
  Synthetic oligonucleotide
gcagctcttgcagcagcagaagttcaactggttgaatcaggcggaggcctggttcaacctggcggatcactgagactgtcatgcgcagcatcaggctttacatttggcaattatgaaatgagctgggttagacaagcacctggcaaaggaccggaatgggtttcaggcgttagccctggcggaggctcaacatattatgcagattcagttaaaggacgcttcatcatttcacgcgataatggcaaaaatacggtctacctgcaaatgaattcactgaaaccggaagatacagcggtctattattgcaatgcagatgtctatacaaatagcggctggcgcaattcatggggacaaggcacacaagttacagtttcaagcggaggcggaagccatcaccatcatcatcattaatctattaaactagtt

SEQ ID NO: 78 - DNA, 438 bp, Artificial Sequence
  Synthetic oligonucleotide
gcagctcttgcagcagcagaagttcaactggttgaatcaggcggaggcctggttcaacctggcggatcactgagactgtcatgcgcagcatcaggctttacattttcatcaacatggatgtattgggtcagacaagcacctggcaaaggcctgaaatgggtttcatcaatttctccggatggcagatcaggctattatgcagattcagttaaaggacgctttacgattagcagagataacgcgaaaaatacggtctacctgcaaatgaattcactgcgtccggaagatacagcagtctattattgcgcagcagcagatccgctgagaggcggatattatgaagatggcatggattacatgggcaaaggcacactggttacagtttcatctggcggaggctcacatcatcaccatcatcattaatctattaaactagtt

SEQ ID NO: 79 - DNA, 432 bp, Artificial Sequence
  Synthetic oligonucleotide
gcagctcttgcagcagcagaagttcaactggttgaatcaggcggaggcctggttcaacctggcggatcactgagactgtcatgcgcagcatcaggctttccgtttggcgcatgctggatgcattgggttagacaagcacctggcaaaggcctggaatgggtttcaacaattaatcctggctcaggcacaatctattattcaccgtcagttaaaggacgctttacaatttcaagcgataatgcggaaaatgtcgtctacctgcaaatgaacaatctgaaagaagaagatacaggcgtctattattgcgcagttgcaccgtatacaacaacagtcgaagatgattatattctgtggggacaaggcacacaagttacagtttcatctggcggaggctcacatcatcaccatcatcattaatctattaaactagtt

SEQ ID NO: 80 - DNA, 435 bp, Artificial Sequence
  Synthetic oligonucleotide
gcagctcttgcagcagcagaagttcaactggttgaatcaggcggaggcctggttcaacctggcggatcactgagactgtcatgcgcagcatcaggctttccgttttcagattcatggatgtattgggttagacaagcacctggcaaaggcctggaatgggtttcatcaattgcaccgtattcaggcacaacgtattatacagattcagtcaaaggacgctttacgattagcagagataatgcgaaaaacacggtctacctgcaaatgaattcactgaaaccggaagatacagcggtctattattgcaatgcaaaatatggccttggctatggcgatccgtatgaatatgattattggggacaaggcacacaagttacagtttcatctggcggaggctcacatcatcaccatcatcattaatctattaaactagtt

SEQ ID NO: 81 - DNA, 31 bp, Artificial Sequence
  Synthetic oligonucleotide
gatccccgggaattcctgttataaaaaaagg

SEQ ID NO: 82 - DNA, 27 bp, Artificial Sequence
  Synthetic oligonucleotide
atgatgttaagaaagaaaacaaagcag

SEQ ID NO: 83 - DNA, 38 bp, Artificial Sequence
  Synthetic oligonucleotide
gaattcccggggatctaagaaaagtgattctgggagag

SEQ ID NO: 84 - DNA, 36 bp, Artificial Sequence
  Synthetic oligonucleotide
ctttcttaacatcatagtagttcaccaccttttccc

SEQ ID NO: 85 - DNA, 25 bp, Artificial Sequence
  Synthetic oligonucleotide
tgctgcaagagctgccggaaataaa

SEQ ID NO: 86 - DNA, 21 bp, Artificial Sequence
  Synthetic oligonucleotide
tctattaaactagttataggg

SEQ ID NO: 87 - DNA, 417 bp, Artificial Sequence
  Synthetic oligonucleotide
gcagctcttgcagcagcagaagttcaactggttgaatcaggcggaggcctggtccaagcaggcggatcactgagactgtcatgcacagcatcagatcagatttttgacaactataacatggcgtggtttagacaatcaccgggaaaagaaagagaatttgttgcagcactgtcatggggagattcaaatacaggctatgcagattcagtcaaaggacgctttacaattagcagagataacgcgaaaaacacggtctatctgcaaatgaattcactgaaaccggaagatacagcggtctattattgctatgcagttacatggctgagaggcgattattggggacaaggcacacaagttacagtttcatctggcggaggctcacatcatcaccatcatcattaatctattaaactagtt

SEQ ID NO: 88 - DNA, 426 bp, Artificial Sequence
  Synthetic oligonucleotide
gcagctcttgcagcagcagaagttcaactggttgaatcaggcggaggcctggttcaacctggcggatcactgacactgtcatgcgcagcatcaggccaaacattttcaagctataatatggcatggtttcgccaatcaccgggaaaagaaagagaatttgttgcgacaatttcatggggaggcggatcaacaggctatgcagattcagttaaaggacgctttacaatctcacgcgatcatgcaaaaaatacggtctacctgcaaatgaaagatctgaaaccggaagatacaggcgcatattattgctatctggttggcctgtttggcattcaagcatcagattattggggacaaggcacacaagttacagtttcatctggcggaggctcacatcatcaccatcatcattaatctattaaactagtt

SEQ ID NO: 89 - DNA, 429 bp, Artificial Sequence
  Synthetic oligonucleotide
gcagctcttgcagcagcagaagttcaactggttgaatcaggcggaggcctggttcaacctggcggatcactgagactgtcatgcgcagcatcaggcacaattttttcaacaaatgcaatgagctggtatagacaagcaccgggaaaacaaagagaactggttgcagcaattacaagcggaggcaatacaaattatgcagattcagtcaaaggacgctttacaattagcagagataacgcgaaaaacacggtctatctgcaaatgaattcactgaaaccggaagatacagcggtctattattgcaatgcacctggcgttgttacaggctcatatgatgttagaaattattggggacaaggcacacaagttacagtttcatctggcggaggctcacatcatcaccatcatcattaatctattaaactagtt

SEQ ID NO: 90 - protein, 135 aa, Artificial Sequence
  Designed peptide
QVQLVESGGGLVQAGGSLRLSCTASDQIFDNYNMAWFRQSPGKEREFVAALSWGDSNTGYADSVKGRFTISRDNAKNTVYLQMNSLKPEDTAVYYCYAVTWLRGDYWGQGTQVTVSSQPKTPKPQSGGSHHHHHH

SEQ ID NO: 91 - protein, 134 aa, Artificial Sequence
  Designed peptide
EVQLVESGGGLVQAGGSLRLSCTASGRTWNIASMTWFRQAPGGKERTFVATIKWSDLATYYTDSVKGRFTISRGNSKNTVYLQMNSLKPEDTGVYFCYAITTGSPLLGGGMDFWGQGTQVTVSSGGGSHHHHHH

SEQ ID NO: 92 - protein, 135 aa, Artificial Sequence
  Designed peptide
QLQLVESGGGLVQAGDSLRLSCTASGRTFSSCAMGWFRQAPGKEREFVAAISRGGGSTSYADSVKGRFTISKDRARNTAYLEMNSLKPEDTAIYYCYAVFPSGGDYWGQGTLVTVSSEPKTPKPQSGGSHHHHHH

SEQ ID NO: 93 - protein, 130 aa, Artificial Sequence
  Designed peptide
QVQLVESGGGLVQPGGSLTLSCAASGQTFSSYNMAWFRQSPGKEREFVATISWGGGSTGYADSVKGRFTISRDHAKNTVYLQMKDLKPEDTGAYYCYLVGLFGIQASDYWGQGTQVTVSSGGGSHHHHHH

SEQ ID NO: 94 - protein, 131 aa, Artificial Sequence
  Designed peptide
ELQLVESGGGLVQPGGSLRLSCAASGTIFSTNAMSWYRQAPGKQRELVAAITSGGNTNYADSVKGRFTISRDNAKNTVYLQMNSLKPEDTAVYYCNAPGVVTGSYDVRNYWGQGTQVTVSSGGGSHHHHHH

SEQ ID NO: 95 - protein, 134 aa, Artificial Sequence
  Designed peptide
AEVQLVESGGGLVQPGGSLRLSCAASGFAFSSYPMYWVRQAPGKGLEWISFIDGEGTSTSYADSVKGRFTISRDNAKNTVYLQMNSLKPEDTAVYYCNALLRRYNYGFTFDNYWGQGTQVTVSSGGGSHHHHHH

SEQ ID NO: 96 - protein, 130 aa, Artificial Sequence
  Designed peptide
AEVQLVESGGGLVQAGDSLRLSCAATRRTSSTYAMGWFRQAPGKGLEWVAAISWDGGRTYYAESVKGRFTISRDNAKNTVYLQMNSLKPEDTAVYYCYSFGGSDFLMDYWGQGTQVTVSSGGGSHHHHHH

SEQ ID NO: 97 - protein, 130 aa, Artificial Sequence
  Designed peptide
AEVQLVESGGGFVQAGGSLRLSCRVSAPTFMTYTMAWFRQAPGNEREFVAALSKNFVTTSYADSVKGRFTISRDNAKNTVYLQMNSLKPEDTAVYYCNVAWSDYEYLEVWGQGTLVTVSSGGGSHHHHHH

SEQ ID NO: 98 - protein, 130 aa, Artificial Sequence
  Designed peptide
AEVQLVESGGDVVQPGGSLRLSCAASGFTFTTYAMTWVRQAPGEGLEAVSTISGADGSTYYADSVKGRFTISRDNANNTVYLQMNSLKPEDTAVYYCAATPWYSASHTYWGQGTQVTVSSGGGSHHHHHH

SEQ ID NO: 99 - protein, 128 aa, Artificial Sequence
  Designed peptide
AEVQLVESGGGLVQAGGSLRLSCTASDQIFDNYNMAWFRQSPGKEREFVAALSWGDSNTGYADSVKGRFTISRDNAKNTVYLQMNSLKPEDTAVYYCYAVTWLRGDYWGQGTQVTVSSGGGSHHHHHH

SEQ ID NO: 100 - protein, 131 aa, Artificial Sequence
  Designed peptide
AEVQLVESGGGLVQPGGSLTLSCAASGQTFSSYNMAWFRQSPGKEREFVATISWGGGSTGYADSVKGRFTISRDHAKNTVYLQMKDLKPEDTGAYYCYLVGLFGIQASDYWGQGTQVTVSSGGGSHHHHHH

SEQ ID NO: 101 - protein, 132 aa, Artificial Sequence
  Designed peptide
AEVQLVESGGGLVQPGGSLRLSCAASGTIFSTNAMSWYRQAPGKQRELVAAITSGGNTNYADSVKGRFTISRDNAKNTVYLQMNSLKPEDTAVYYCNAPGVVTGSYDVRNYWGQGTQVTVSSGGGSHHHHHH

SEQ ID NO: 102 - protein, 135 aa, Artificial Sequence
  Designed peptide
AEVQLVESGGGLVQAGGSLRLSCTASGRTWNIASMTWFRQAPGGKERTFVATIKWSDLATYYTDSVKGRFTISRGNSKNTVYLQMNSLKPEDTGVYFCYAITTGSPLLGGGMDFWGKGTLVTVSSGGGSHHHHHH

SEQ ID NO: 103 - protein, 128 aa, Artificial Sequence
  Designed peptide
AEVQLVESGGGLVQAGDSLRLSCTASGRTFSSCAMGWFRQAPGKEREFVAAISRGGGSTSYADSVKGRFTISKDRARNTAYLEMNSLKPEDTAIYYCYAVFPSGGDYWGQGTQVTVSSGGGSHHHHHH

SEQ ID NO: 104 - DNA, 438 bp, Artificial Sequence
  Synthetic oligonucleotide
gcagctcttgcagcagcagaagttcaactggttgaatcaggcggaggcctggtccaagcaggcggatcactgagactgtcatgcacagcatcaggcagaacatggaatattgcatcaatgacatggtttagacaagcacctggcggaaaagaaagaacatttgttgcgacaatcaaatggtcagatctggcgacatattatacggattcagtcaaaggacgctttacaatttcaagaggcaacagcaaaaacacggtctatctgcaaatgaattcactgaaaccggaagatacaggcgtctatttttgctatgcaattacaacaggctcaccgctgcttggcggaggcatggatttttggggcaaaggcacactggttacagtttcaagcggaggcggaagccatcaccatcatcatcattaatctattaaactagtt

SEQ ID NO: 105 - DNA, 417 bp, Artificial Sequence
  Synthetic oligonucleotide
gcagctcttgcagcagcagaagttcaactggttgaatcaggcggaggcctggttcaagcaggcgattcactgagactgtcatgcacagcatcaggcagaacattttcatcatgcgcaatgggctggtttagacaagcaccgggaaaagaaagagaatttgttgcagcaatttcaagaggcggaggatcaacatcatatgcagattcagttaaaggacgcttcacgatttcaaaagatagagcaagaaatacggcgtatctggaaatgaattcactgaaaccggaagatacggcgatctattattgctatgcagtttttccgagcggaggcgattattggggacaaggcacacaagttacagtttcatctggcggaggctcacaccatcatcatcaccattaatctattaaactagtt

SEQ ID NO: 106 - protein, 121 aa, Artificial Sequence
  Designed peptide
EVQLVESGGGLVQPGGSLRLSCAASGTIFSTNAMSWYRQAPGKQRELVAAITSGGNTNYADSVKGRFTISRDNAKNTVYLQMNSLKPEDTAVYYCNAPGVVTGSYDVKNYWGQGTQVTVSS

SEQ ID NO: 107 - protein, 121 aa, Artificial Sequence
  Designed peptide
EVQLVESGGGLVQPGGSLRLSCAASGTIFSTNAMSWYRQAPGKQRELVAAITSGGNTNYADSVKGRFTISRDNAKNTVYLQMNSLKPEDTAVYYCNAPGVVTGSYDVRDYWGQGTQVTVSS

SEQ ID NO: 108 - protein, 121 aa, Artificial Sequence
  Designed peptide
EVQLVESGGGLVQPGGSLRLSCAASGTIFSTNAMSWYRQAPGKQRELVAAITSGGNTNYADSVKGRFTISRDNAKNTVYLQMNSLKPEDTAVYYCNAPGVVTGSYDVRNSWGQGTQVTVSS

SEQ ID NO: 109 - protein, 130 aa, Artificial Sequence
  Designed peptide
AEVQLVESGGGLVQPGGSLRLSCAASGTIFSTNAMSWYRQAPGKQRELVAAITSGGNTNYADSVKGRFTISRDNAKNTVYLQMNSLKPEDTAVYYCNAPGVVTGSYDVKNYWGQGTQVTVSSGSHHHHHH

SEQ ID NO: 110 - protein, 130 aa, Artificial Sequence
  Designed peptide
AEVQLVESGGGLVQPGGSLRLSCAASGTIFSTNAMSWYRQAPGKQRELVAAITSGGNTNYADSVKGRFTISRDNAKNTVYLQMNSLKPEDTAVYYCNAPGVVTGSYDVRDYWGQGTQVTVSSGSHHHHHH

SEQ ID NO: 111 - protein, 130 aa, Artificial Sequence
  Designed peptide
AEVQLVESGGGLVQPGGSLRLSCAASGTIFSTNAMSWYRQAPGKQRELVAAITSGGNTNYADSVKGRFTISRDNAKNTVYLQMNSLKPEDTAVYYCNAPGVVTGSYDVRNSWGQGTQVTVSSGSHHHHHH